European Patent Application EP 4 538 296 A1, published April 16, 2025. Title: GLYCOSYL-MODIFIED FUSION PROTEIN, NUCLEIC ACID MOLECULE, EXPRESSION VECTOR, HOST CELL AND APPLICATIONS THEREOF. Applicant: Kaimi Biomedicine (Chengdu) Co., Ltd. Application EP. The sequence listing filed with the application follows.

SEQUENCE LISTING (7 sequences)

SEQ ID NO: 1 - protein, 232 aa, Mus musculus
VDKKIVPRDCGCKPCICTVPEVSSVFIFPPKPKDVLTITLTPKVTCVVVDISKDDPEVQFSWFVDDVEVHTAQTQPREEQFNSTFRSVSELPIMHQDWLNGKEFKCRVNSAAFPAPIEKTISKTKGRPKAPQVYTIPPPKEQMAKDKVSLTCMITDFFPEDITVEWQWNGQPAENYKNTQPIMDTDGSYFVYSKLNVQKSNWEAGNTFTCSVLHEGLHNHHTEKSLSHSPGL

SEQ ID NO: 2 - protein, 232 aa, synthetic construct
VDKKIVPADCGCAPCICAVPEVSSVFIFPPKPKDVLTITLTPKVTCVVVDISKDDPEVQFSWFVDDVEVHTAQTQPREEQFNSTFRSVSELPIMHQDWLNGKEFKCRVNSAAFPAPIEKTISKTKGRPKAPQVYTIPPPKEQMAKDKVSLTCMITDFFPEDITVEWQWNGQPAENYKNTQPIMDTDGSYFVYSKLNVQKSNWEAGNTFTCSVLHEGLHNHHTEKSLSHSPGL

SEQ ID NO: 3 - protein, 232 aa, synthetic construct
VDKKIVPADCGCAPCICAVPEVSSVFIFPPKPKDVLTITLTPKVTCVVVDISKDDPEVQFSWFVDDVEVHTAQTQPREEQFNSTFRSVSELPIMHQDWLNGKEFKCRVNSAAFPLPEEKTISKTKGRPKAPQVYTIPPPKEQMAKDKVSLTCMITDFFPEDITVEWQWNGQPAENYKNTQPIMDTDGSYFVYSKLNVQKSNWEAGNTFTCSVLHEGLHNHHTEKSLSHSPGL

SEQ ID NO: 4 - protein, 644 aa, synthetic construct
SYYHHHHHHDYDIPTTENLYFQGAMDPEFKGLRRRMKKWSSKPRKGMGTNLSVPNPLGFFPDHQLDPVFGANSNNPDWDFNPIKDHWPAANQVGVGAFGPGFTPPHGGVLGWSPQAQGMLTPVSTIPPPASANRQSGRQPTPISPPLRDSHPQAMQWNSTAFHQALQDPRVRGLYFPAGGSSSGTVNPAPNIASHISSISARTGDPVTNMDIDPYKEFGATVELLSFLPSDFFPSVRDLLDTASALYREALESPEHCSPHHTALRQAILCWGELMTLATWVGNNLEDPASRDLVVNYVNTNMGLKIRQLLWFHISCLTFGRETVLEYLVSFGVWIRTPPAYRPPNAPILSTLPETTVVRRRDRGRSPRRRTPSPRRRRSQSPRRRRSQSRESQCVRPQGGGSVDKKIVPADCGCAPCICAVPEVSSVFIFPPKPKDVLTITLTPKVTCVVVDISKDDPEVQFSWFVDDVEVHTAQTQPREEQFNSTFRSVSELPIMHQDWLNGKEFKCRVNSAAFPAPIEKTISKTKGRPKAPQVYTIPPPKEQMAKDKVSLTCMITDFFPEDITVEWQWNGQPAENYKNTQPIMDTDGSYFVYSKLNVQKSNWEAGNTFTCSVLHEGLHNHHTEKSLSHSPGLQSLSRSTRGS

SEQ ID NO: 5 - protein, 592 aa, synthetic construct
KELKFVTLVFRHGDRSPIDTFPTDPIKESSWPQGFGQLTQLGMEQHYELGEYIRKRYRKFLNESYKHEQVYIRSTDVDRTLMSAMTNLAALFPPEGVSIWNPILLWQPIPVHTVPLSEDQLLYLPFRNCPRFQELESETLKSEEFQKRLHPYKDFIATLGKLSGLHGQDLFGIWSKVYDPLYCESVHNFTLPSWATEDTMTKLRELSELSLLSLYGIHKQKEKSRLQGGVLVNEILNHMKRATQIPSYKKLIMYSAHDTTVSGLQMALDVYNGLLPPYASCHLTELYFEKGEYFVEMYYRNETQHEPYPLMLPGCSPSCPLERFAELVGPVIPQDWSTECMTTNSHQGTEDSTDSRGGGSVDKKIVPADCGCAPCICAVPEVSSVFIFPPKPKDVLTITLTPKVTCVVVDISKDDPEVQFSWFVDDVEVHTAQTQPREEQFNSTFRSVSELPIMHQDWLNGKEFKCRVNSAAFPAPIEKTISKTKGRPKAPQVYTIPPPKEQMAKDKVSLTCMITDFFPEDITVEWQWNGQPAENYKNTQPIMDTDGSYFVYSKLNVQKSNWEAGNTFTCSVLHEGLHNHHTEKSLSHSPGL

SEQ ID NO: 6 - protein, 592 aa, synthetic construct
KELKFVTLVFRHGDRSPIDTFPTDPIKESSWPQGFGQLTQLGMEQHYELGEYIRKRYRKFLNESYKHEQVYIRSTDVDRTLMSAMTNLAALFPPEGVSIWNPILLWQPIPVHTVPLSEDQLLYLPFRNCPRFQELESETLKSEEFQKRLHPYKDFIATLGKLSGLHGQDLFGIWSKVYDPLYCESVHNFTLPSWATEDTMTKLRELSELSLLSLYGIHKQKEKSRLQGGVLVNEILNHMKRATQIPSYKKLIMYSAHDTTVSGLQMALDVYNGLLPPYASCHLTELYFEKGEYFVEMYYRNETQHEPYPLMLPGCSPSCPLERFAELVGPVIPQDWSTECMTTNSHQGTEDSTDSRGGGSVDKKIVPADCGCAPCICAVPEVSSVFIFPPKPKDVLTITLTPKVTCVVVDISKDDPEVQFSWFVDDVEVHTAQTQPREEQFNSTFRSVSELPIMHQDWLNGKEFKCRVNSAAFPLPEEKTISKTKGRPKAPQVYTIPPPKEQMAKDKVSLTCMITDFFPEDITVEWQWNGQPAENYKNTQPIMDTDGSYFVYSKLNVQKSNWEAGNTFTCSVLHEGLHNHHTEKSLSHSPGL

SEQ ID NO: 7 - protein, 597 aa, synthetic construct
KELKFVTLVFRHGDRSPIDTFPTDPIKESSWPQGFGQLTQLGMEQHYELGEYIRKRYRKFLNESYKHEQVYIRSTDVDRTLMSAMTNLAALFPPEGVSIWNPILLWQPIPVHTVPLSEDQLLYLPFRNCPRFQELESETLKSEEFQKRLHPYKDFIATLGKLSGLHGQDLFGIWSKVYDPLYCESVHNFTLPSWATEDTMTKLRELSELSLLSLYGIHKQKEKSRLQGGVLVNEILNHMKRATQIPSYKKLIMYSAHDTTVSGLQMALDVYNGLLPPYASCHLTELYFEKGEYFVEMYYRNETQHEPYPLMLPGCSPSCPLERFAELVGPVIPQDWSTECMTTNSHQGTEDSTDSRGGGSVDKRVEPKSCDKTHTCPPCPAPELLGGPSVFLFPPKPKDTLMISRTPEVTCVVVDVSHEDPEVKFNWYVDGVEVHNAKTKPREEQYNSTYRVVSVLTVLHQDWLNGKEYKCKVSNKALPAPIEKTISKAKGQPREPQVYTLPPSREEMTKNQVSLTCLVKGFYPSDIAVEWESNGQPENNYKTTPPVLDSDGSFFLYSKLTVDKSRWQQGNVFSCSVMHEALHNHYTQKSLSLSPGK